European Patent Application EP 4 635 970 A1, published October 22, 2025. Title: synthetic peptide and construct. Applicant: TOAGOSEI CO., LTD. The sequence listing filed with the application follows.

SEQUENCE LISTING (14 sequences)

SEQ ID NO: 1 - protein, 4 aa, synthetic construct
GDGD

SEQ ID NO: 2 - protein, 4 aa, synthetic construct
GEGE

SEQ ID NO: 3 - protein, 4 aa, synthetic construct
GDGE

SEQ ID NO: 4 - protein, 4 aa, synthetic construct
GEGD

SEQ ID NO: 5 - protein, 5 aa, synthetic construct
GDGDG

SEQ ID NO: 6 - protein, 5 aa, synthetic construct
GEGEG

SEQ ID NO: 7 - protein, 5 aa, synthetic construct
GDGEG

SEQ ID NO: 8 - protein, 5 aa, synthetic construct
GEGDG

SEQ ID NO: 9 - protein, 7 aa, synthetic construct
GDGDGDG

SEQ ID NO: 10 - protein, 9 aa, synthetic construct
GDGDGDGDG

SEQ ID NO: 11 - protein, 11 aa, synthetic construct
GDGDGDGDGDG

SEQ ID NO: 12 - protein, 13 aa, synthetic construct
GDGDGDGDGDGDG

SEQ ID NO: 13 - protein, 13 aa, synthetic construct
GEGEGEGEGEGEG

SEQ ID NO: 14 - protein, 13 aa, synthetic construct
GDGEGDGEGDGEG